European Patent Application EP 4 647 496 A1, published November 12, 2025. Title: A novel promoter and use thereof. Applicant: CJ CheilJedang Corporation. The sequence listing filed with the application follows.

SEQUENCE LISTING (15 sequences)

SEQ ID NO: 1 - DNA, 125 bp, synthetic construct
  misc_feature 1..125: note = Psba
  source 1..125: mol_type = other DNA
gatttttgatggacgaaatctggatggggtggtagcgtagtggctgcactgtcatcgcacgatagcatcggttcgcgtgcccagtgcttcgacagttacatagattattggaggagatcaaaaca

SEQ ID NO: 2 - DNA, 125 bp, synthetic construct
  misc_feature 1..125: note = Psbb
  source 1..125: mol_type = other DNA
acactctgatcgtcggagtcattttcgaataatcccaggtccattgtccagaacggtggtgatctgcgctgatgcgaaatagtcgctatcatggcgggtgaagacacgagaaggaaggttcatag

SEQ ID NO: 3 - DNA, 125 bp, synthetic construct
  misc_feature 1..125: note = Psbc
  source 1..125: mol_type = other DNA
cctcctccactgtcatgcttttcagcaattgatttgcttgcccaaccccgatagaggtaaattaactttaatttaaacacccgagttagggtaggagtcagaactagaagaagaaggtcggtgaa

SEQ ID NO: 4 - DNA, 720 bp, synthetic construct
  misc_feature 1..720: note = eGFP
  source 1..720: mol_type = other DNA
atggtgagcaagggcgaggagctgttcaccggggtggtgcccatcctggtcgagctggacggcgacgtaaacggccacaagttcagcgtgtccggcgagggcgagggcgatgccacctacggcaagctgaccctgaagttcatctgcaccaccggcaagctgcccgtgccctggcccaccctcgtgaccaccctgacctacggcgtgcagtgcttcagccgctaccccgaccacatgaagcagcacgacttcttcaagtccgccatgcccgaaggctacgtccaggagcgcaccatcttcttcaaggacgacggcaactacaagacccgcgccgaggtgaagttcgagggcgacaccctggtgaaccgcatcgagctgaagggcatcgacttcaaggaggacggcaacatcctggggcacaagctggagtacaactacaacagccacaacgtctatatcatggccgacaagcagaagaacggcatcaaggtgaacttcaagatccgccacaacatcgaggacggcagcgtgcagctcgccgaccactaccagcagaacacccccatcggcgacggccccgtgctgctgcccgacaaccactacctgagcacccagtccgccctgagcaaagaccccaacgagaagcgcgatcacatggtcctgctggagttcgtgaccgccgccgggatcactctcggcatggacgagctgtacaagtaa

SEQ ID NO: 5 - DNA, 43 bp, synthetic construct
  misc_feature 1..43: note = primer
  source 1..43: mol_type = other DNA
acggtatcgataagcttgatatcatggtgagcaagggcgagga

SEQ ID NO: 6 - DNA, 40 bp, synthetic construct
  misc_feature 1..40: note = primer
  source 1..40: mol_type = other DNA
ccgggctgcaggaattcgatttacttgtacagctcgtcca

SEQ ID NO: 7 - DNA, 40 bp, synthetic construct
  misc_feature 1..40: note = primer
  source 1..40: mol_type = other DNA
acggtatcgataagcttgatagaaacatcccagcgctact

SEQ ID NO: 8 - DNA, 40 bp, synthetic construct
  misc_feature 1..40: note = primer
  source 1..40: mol_type = other DNA
tcgcccttgctcaccatgatgagtgtttcctttcgttggg

SEQ ID NO: 9 - DNA, 40 bp, synthetic construct
  misc_feature 1..40: note = primer
  source 1..40: mol_type = other DNA
acggtatcgataagcttgatgatttttgatggacgaaatc

SEQ ID NO: 10 - DNA, 40 bp, synthetic construct
  misc_feature 1..40: note = primer
  source 1..40: mol_type = other DNA
tcgcccttgctcaccatgattgttttgatctcctccaata

SEQ ID NO: 11 - DNA, 40 bp, synthetic construct
  misc_feature 1..40: note = primer
  source 1..40: mol_type = other DNA
acggtatcgataagcttgatacactctgatcgtcggagtc

SEQ ID NO: 12 - DNA, 40 bp, synthetic construct
  misc_feature 1..40: note = primer
  source 1..40: mol_type = other DNA
tcgcccttgctcaccatgatctatgaaccttccttctcgt

SEQ ID NO: 13 - DNA, 40 bp, synthetic construct
  misc_feature 1..40: note = primer
  source 1..40: mol_type = other DNA
acggtatcgataagcttgatcctcctccactgtcatgctt

SEQ ID NO: 14 - DNA, 40 bp, synthetic construct
  misc_feature 1..40: note = primer
  source 1..40: mol_type = other DNA
tcgcccttgctcaccatgatttcaccgaccttcttcttct

SEQ ID NO: 15 - DNA, 318 bp, synthetic construct
  misc_feature 1..318: note = Pcj7
  source 1..318: mol_type = other DNA
agaaacatcccagcgctactaatagggagcgttgaccttccttccacggaccggtaatcggagtgcctaaaaccgcatgcggcttaggctccaagataggttctgcgcggccgggtaatgcatcttctttagcaacaagttgaggggtaggtgcaaataagaacgacatagaaatcgtctcctttctgtttttaatcaacatacaccaccacctaaaaattccccgaccagcaagttcacagtattcgggcacaatatcgttgccaaaatattgtttcggaatatcatgggatacgtacccaacgaaaggaaacactc